European Patent Application EP 4 700 128 A1, published February 25, 2026. Title: Microbial oil composition comprising retinoid and fatty acid. Applicant: 씨제이제일제당 주식회사. The sequence listing filed with the application follows.

SEQUENCE LISTING (8 sequences)

SEQ ID NO: 1 - protein, 673 aa, Xanthophyllomyces dendrorhous
MTALAYYQIHLIYTLPILGLLGLLTSPILTKFDIYKISILVFIAFSATTPWDSWIIRNGAWTYPSAESGQGVFGTFLDVPYEEYAFFVIQTVITGLVYVLATRHLLPSLALPKTRSSALSLALKALIPLPIIYLFTAHPSPSPDPLVTDHYFYMRALSLLITPPTMLLAALSGEYAFDWKSGRAKSTIAAIMIPTVYLIWVDYVAVGQDSWSINDEKIVGWRLGGVLPIEEAMFFLLTNLMIVLGLSACDHTQALYLLHGRTIYGNKKMPSSFPLITPPVLSLFFSSRPYSSQPKRDLELAVKLLEEKSRSFFVASAGFPSEVRERLVGLYAFCRVTDDLIDSPEVSSNPHATIDMVSDFLTLLFGPPLHPSQPDKILSSPLLPPSHPSRPTGMYPLPPPPSLSPAELVQFLTERVPVQYHFAFRLLAKLQGLIPRYPLDELLRGYTTDLIFPLSTEAVQARKTPIETTADLLDYGLCVAGSVAELLVYVSWASAPSQVPATIEEREAVLVASREMGTALQLVNIARDIKGDATEGRFYLPLSFFGLRDESKLAIPTDWTEPRPQDFDKLLSLSPSSTLPSSNASESFRFEWKTYSLPLVAYAEDLAKHSYKGIDRLPTEVQAGMRAACASYLLIGREIKVVWKGDVGERRTVAGWRRVRKVLSVVMSGWEGQ

SEQ ID NO: 2 - DNA, 2022 bp, Xanthophyllomyces dendrorhous
  source 1..2022: mol_type = genomic DNA
atgacggctctcgcatattaccagatccatctgatctatactctcccaattcttggtcttctcggcctgctcacttccccgattttgacaaaatttgacatctacaaaatatcgatcctcgtatttattgcgtttagtgcaaccacaccatgggactcatggatcatcagaaatggcgcatggacatatccatcagcggagagtggccaaggcgtgtttggaacgtttctagatgttccatatgaagagtacgctttctttgtcattcaaaccgtaatcaccggcttggtctacgtcttggcaactaggcaccttctcccatctctcgcgcttcccaagactagatcgtccgccctttctctcgcgctcaaggcgctcatccctctgcccattatctacctatttaccgctcaccccagcccatcgcccgacccgctcgtgacagatcactacttctacatgcgggcactctccttactcatcaccccacctaccatgctcttggcagcattatcaggcgaatatgctttcgattggaaaagtggccgagcaaagtcaactattgcagcaatcatgatcccgacggtgtatctgatttgggtagattatgttgctgtcggtcaagactcttggtcgatcaacgatgagaagattgtagggtggaggcttggaggtgtactacccattgaggaagctatgttcttcttactgacgaatctaatgattgttctgggtctgtctgcctgcgatcatactcaggccctatacctgctacacggtcgaactatttatggcaacaaaaagatgccatcttcatttcccctcattacaccgcctgtgctctccctgttttttagcagccgaccatactcttctcagccaaaacgtgacttggaactggcagtcaagttgttggaggaaaagagccggagcttttttgttgcctcggctggatttcctagcgaagttagggagaggctggttggactatacgcattctgccgggtgactgatgatcttatcgactctcctgaagtatcttccaacccgcatgccacaattgacatggtctccgattttcttaccctactatttgggcccccgctacacccttcgcaacctgacaagatcctttcttcgcctttacttcctccttcgcacccttcccgacccacgggaatgtatcccctcccgcctcctccttcgctctcgcctgccgagctcgttcaattccttaccgaaagggttcccgttcaataccatttcgccttcaggttgctcgctaagttgcaagggctgatccctcgatacccactcgacgaactccttagaggatacaccactgatcttatctttcccttatcgacagaggcagtccaggctcggaagacgcctatcgagaccacagctgacttgctggactatggtctatgtgtagcaggctcagtcgccgagctattggtctatgtctcttgggcaagtgcaccaagtcaggtccctgccaccatagaagaaagagaagctgtgttagtggcaagccgagagatgggaactgcccttcagttggtgaacattgctagggacattaaaggggacgcaacagaagggagattttacctaccactctcattctttggtcttcgggatgaatcaaagcttgcgatcccgactgattggacggaacctcggcctcaagatttcgacaaactcctcagtctatctccttcgtccacattaccatcttcaaacgcctcagaaagcttccggttcgaatggaagacgtactcgcttccattagtcgcctacgcagaggatcttgccaaacattcttataagggaattgaccgacttcctaccgaggttcaagcgggaatgcgagcggcttgcgcgagctacctactgatcggccgagagatcaaagtcgtttggaaaggagacgtcggagagagaaggacagttgccggatggaggagagtacggaaagtcttgagtgtggtcatgagcggatgggaagggcagtaa

SEQ ID NO: 3 - protein, 582 aa, Xanthophyllomyces dendrorhous
MGKEQDQDKPTAIIVGCGIGGIATAARLAKEGFQVTVFEKNDYSGGRCSLIERDGYRFDQGPSLLLLPDLFKQTFEDLGEKMEDWVDLIKCEPNYVCHFHDEETFTLSTDMALLKREVERFEGKDGFDRFLSFIQEAHRHYELAVVHVLQKNFPGFAAFLRLQFIGQILALHPFESIWTRVCRYFKTDRLRRVFSFAVMYMGQSPYSAPGTYSLLQYTELTEGIWYPRGGFWQVPNTLLQIVKRNNPSAKFNFNAPVSQVLLSPAKDRATGVRLESGEEHHADVVIVNADLVYASEHLIPDDARNKIGQLGEVKRSWWADLVGGKKLKGSCSSLSFYWSMDRIVDGLGGHNIFLAEDFKGSFDTIFEELGLPADPSFYVNVPSRIDPSAAPEGKDAIVILVPCGHIDASNPQDYNKLVARARKFVIHTLSAKLGLPDFEKMIVAEKVHDAPSWEKEFNLKDGSILGLAHNFMQVLGFRPSTRHPKYDKLFFVGASTHPGTGVPIVLAGAKLTANQVLESFDRSPAPDPNMSLSVPYGKPLKSNGTGIDSQVQLKFMDLERWVYLLVLLIGAVIARSVGVLAF

SEQ ID NO: 4 - DNA, 1749 bp, Xanthophyllomyces dendrorhous
  source 1..1749: mol_type = genomic DNA
atgggaaaagaacaagatcaggataaacccacagctatcatcgtgggatgtggtatcggtggaatcgccactgccgctcgtcttgctaaagaaggtttccaggtcacggtgttcgagaagaacgactactccggaggtcgatgctctttaatcgagcgagatggttatcgattcgatcaggggcccagtttgctgctcttgccagatctcttcaagcagacattcgaagatttgggagagaagatggaagattgggtcgatctcatcaagtgtgaacccaactatgtttgccacttccacgatgaagagactttcactctttcaaccgacatggcgttgctcaagcgggaagtcgagcgttttgaaggcaaagatggatttgatcggttcttgtcgtttatccaagaagcccacagacattacgagcttgctgtcgttcacgtcctgcagaagaacttccctggcttcgcagcattcttacggctacagttcattggccaaatcctggctcttcaccccttcgagtctatctggacaagagtttgtcgatatttcaagaccgacagattacgaagagtcttctcgtttgcagtgatgtacatgggtcaaagcccatacagtgcgcccggaacatattccttgctccaatacaccgaattgaccgagggcatctggtatccgagaggaggcttttggcaggttcctaatactcttcttcagatcgtcaagcgcaacaatccctcagccaagttcaatttcaacgctccagtttcccaggttcttctctctcctgccaaggaccgagcgactggtgttcgacttgaatccggcgaggaacatcacgccgatgttgtgattgtcaatgctgacctcgtttacgcctccgagcacttgattcctgacgatgccagaaacaagattggccaactgggtgaagtcaagagaagttggtgggctgacttagttggtggaaagaagctcaagggaagttgcagtagtttgagcttctactggagcatggaccgaatcgtggacggtctgggcggacacaatatcttcttggccgaggacttcaagggatcattcgacacaatcttcgaggagttgggtctcccagccgatccttccttttacgtgaacgttccctcgcgaatcgatccttctgccgctcccgaaggcaaagatgctatcgtcattcttgtgccgtgtggccatatcgacgcttcgaaccctcaagattacaacaagcttgttgctcgggcaaggaagtttgtgatccacacgctttccgccaagcttggacttcccgactttgaaaaaatgattgtggcagagaaggttcacgatgctccctcttgggagaaagaattcaacctcaaggacggaagcatcttgggactggctcacaactttatgcaagttcttggtttcaggccgagcaccagacatcccaagtatgacaagttgttctttgtcggggcttcgactcatcccggaactggggttcccatcgtcttggctggagccaagttaactgccaaccaagttctcgaatcctttgaccgatccccagctccagatcccaatatgtcactctccgtaccatatggaaaacctctcaaatcaaatggaacgggtatcgattctcaggtccagctgaagttcatggatttggagagatgggtataccttttggtgttgttgattggggccgtgatcgctcgatccgttggtgttcttgctttctga

SEQ ID NO: 5 - protein, 338 aa, Haematococcus pluvialis
MIRAMHNRAPTPRTRVSHPRSHRALAHVSAVATAGQVAEVHSAPAFDFEMYMRDRAEMVNKALDAALPSRYPEVLVDSMRYSVLAGGKRVRPALTLAACDLVGGDMATALPTACAMEMIHTMSLIHDDLPAMDNDDFRRGRPTNHKVYGEDIAILAGDALLSFAFEHIARDTKGVPADAVLKVIMELGRAVGAQGLSAGQAVDIKSEGQEVGLEVLEYIHHHKTAALLEAAVVCGALVGGADTATVEKLRKYALNIGLAFQVIDDILDVTQTTETLGKTAAKDLAVNKTTYPKLLGLEASRKVADDLIREAIAQLDEFEPARKAPMVALAHLIGYRKN

SEQ ID NO: 6 - DNA, 1017 bp, Haematococcus pluvialis
  source 1..1017: mol_type = genomic DNA
atgatccgagcgatgcacaaccgggcgcccacacctcgaactcgagtgtctcatccacgctcacatagggctctggcacatgtctcagccgtagcaacagcagggcaggtggcagaggtccactctgctcctgcctttgacttcgagatgtacatgagagacagagctgagatggtcaacaaggctcttgatgctgcattgccatctagataccctgaggtgctggttgattccatgaggtactccgtacttgcgggtggcaagcgcgtgaggcctgccctgacactggctgcgtgcgaccttgtaggaggggacatggccactgccctacccaccgcatgtgccatggagatgatccacaccatgagcctcatccatgatgacctgccagccatggacaatgacgacttcaggcgaggtcggcccacaaaccataaggtgtatggtgaggacattgccatccttgctggtgacgcgctgctgtcctttgcctttgagcacatcgcccgggacaccaaaggcgtgccggctgatgcggtgctgaaggtcatcatggagctgggccgggccgtgggcgcgcagggcctatcagcaggccaggctgttgacataaagagcgagggccaggaggtggggctggaggtgctggagtacatccaccaccacaagacagctgcactgctggaggcggcagtggtgtgcggcgcactggtgggcggggccgacaccgccaccgtggagaagctgcgcaagtacgcgctgaacattgggctggccttccaggtgattgatgacatcctggacgtcactcaaaccaccgaaaccttgggcaagaccgcagccaaagacctggcggtgaacaagaccacctatcccaagctgctgggtctggaagccagcaggaaggtggcggacgacttgatcagggaggctatagcacagttagacgagtttgagcctgcacgcaaggcgcccatggtggccctggcccacctcatagggtaccgcaagaactga

SEQ ID NO: 7 - protein, 275 aa, Marinebacterium [sequence omitted]

SEQ ID NO: 8 - DNA, 828 bp, Marinebacterium
  source 1..828: mol_type = genomic DNA
atgggcctgatgctgatcgactggtgtgccctggccctggtggtgttcatcggcctgccccacggcgccctggacgccgccatctctttctctatgatctcttctgccaagcgaatcgcccgactggccggcatcctgctgatctacctgctgctggccaccgccttcttcctgatctggtaccagctgcccgccttctctctgctgatcttcctgctgatctctatcatccacttcggcatggccgacttcaacgcctctccctctaagctgaagtggccccacatcatcgcccacggcggcgtggtgaccgtgtggctgcccctgatccagaagaacgaggtgaccaagctgttctctatcctgaccaacggccccacccccatcctgtgggacatcctgctgatcttcttcctgtgttggtctatcggcgtgtgtctgcacacctacgagaccctgcgatctaagcactacaacatcgccttcgagctgatcggcctgatcttcctggcctggtacgccccccccctggtgaccttcgccacctacttctgtttcatccactctcgacgacacttctctttcgtgtggaagcagctgcagcacatgtcttctaagaagatgatgatcggctctgccatcatcctgtcttgtacctcttggctgatcggcggcggcatctacttcttcctgaactctaagatgatcgcctctgaggccgccctgcagaccgtgttcatcggcctggccgccctgaccgtgccccacatgatcctgatcgacttcatcttccgaccccactcttctcgaatcaagatcaagaactag